European Patent Application EP 4 582 443 A1, published July 9, 2025. Title: RECOMBINANT HUMAN ALBUMIN EXPRESSION LEVEL IMPROVING METHOD AND CELLS AND PROTEINS. Applicant: TONGHUA ANRATE BIOPHARMACEUTICAL CO., LTD. The sequence listing filed with the application follows.

SEQUENCE LISTING (17 sequences)

SEQ ID NO: 1 - DNA, 267 bp, synthetic construct
  source 1..267: mol_type = other DNA
atgagattcccatctattttcaccgctgtcttgttcgctgcctcctctgcattggctgcccctgttaacactaccactgaagacgagactgctcaaattccagctgaagcagttatcggttactctgaccttgagggtgatttcgacgtcgctgttttgcctttctctaactccactaacaacggtttgttgttcattaacaccactatcgcttccattgctgctaaggaagagggtgtctctctcgagaagagagaggccgaagct

SEQ ID NO: 2 - DNA, 72 bp, synthetic construct
  source 1..72: mol_type = other DNA
atgaagtgggtaacctttatttcccttctttttctctttagctcggcttattccaggggtgtgtttcgtcga

SEQ ID NO: 3 - DNA, 1758 bp, synthetic construct
  source 1..1758: mol_type = other DNA
gatgcacacaagagtgaggttgctcatcggtttaaagatttgggagaagaaaatttcaaagccttggtgttgattgcctttgctcagtatcttcagcagtgtccatttgaagatcatgtaaaattagtgaatgaagtaactgaatttgcaaaaacatgtgttgctgatgagtcagctgaaaattgtgacaaatcacttcataccctttttggagacaaattatgcacagttgcaactcttcgtgaaacctatggtgaaatggctgactgctgtgcaaaacaagaacctgagagaaatgaatgcttcttgcaacacaaagatgacaacccaaacctcccccgattggtgagaccagaggttgatgtgatgtgcactgcttttcatgacaatgaagagacatttttgaaaaaatacttatatgaaattgccagaagacatccttacttttatgccccggaactccttttctttgctaaaaggtataaagctgcttttacagaatgttgccaagctgctgataaagctgcctgcctgttgccaaagctcgatgaacttcgggatgaagggaaggcttcgtctgccaaacagagactcaagtgtgccagtctccaaaaatttggagaaagagctttcaaagcatgggcagtagctcgcctgagccagagatttcccaaagctgagtttgcagaagtttccaagttagtgacagatcttaccaaagtccacacggaatgctgccatggagatctgcttgaatgtgctgatgacagggcggaccttgccaagtatatctgtgaaaatcaagattcgatctccagtaaactgaaggaatgctgtgaaaaacctctgttggaaaaatcccactgcattgccgaagtggaaaatgatgagatgcctgctgacttgccttcattagctgctgattttgttgaaagtaaggatgtttgcaaaaactatgctgaggcaaaggatgtcttcctgggcatgtttttgtatgaatatgcaagaaggcatcctgattactctgtcgtgctgctgctgagacttgccaagacatatgaaaccactctagagaagtgctgtgccgctgcagatcctcatgaatgctatgccaaagtgttcgatgaatttaaacctcttgtggaagagcctcagaatttaatcaaacaaaattgtgagctttttgagcagcttggagagtacaaattccagaatgcgctattagttcgttacaccaagaaagtaccccaagtgtcaactccaactcttgtagaggtctcaagaaacctaggaaaagtgggcagcaaatgttgtaaacatcctgaagcaaaaagaatgccctgtgcagaagactatctatccgtggtcctgaaccagttatgtgtgttgcatgagaaaacgccagtaagtgacagagtcaccaaatgctgcacagaatccttggtgaacaggcgaccatgcttttcagctctggaagtcgatgaaacatacgttcccaaagagtttaatgctgaaacattcaccttccatgcagatatatgcacactttctgagaaggagagacaaatcaagaaacaaactgcacttgttgagctcgtgaaacacaagcccaaggcaacaaaagagcaactgaaagctgttatggatgatttcgcagcttttgtagagaagtgctgcaaggctgacgataaggagacctgctttgccgaggagggtaaaaaacttgttgctgcaagtcaagctgccttaggcttataa

SEQ ID NO: 4 - DNA, 465 bp, synthetic construct
  source 1..465: mol_type = other DNA
atggtcaaagcagttgcagtcttaagaggcgattctaccgtcggcggtaccgttgtcttcgaacaatcctccgaaagcagccctaccactatcacttacgacatcaaaggtaactccccaaacgctgagagaggtttccacattcaccagttcggtgacaataccaatggttgtacttcagctggtcctcacttcaacccatttggtaagacccacggtgctccaactgacgaagctagacacgtcggtgacttgggtaacgtcaagaccgacgctgaaggtgttgccaagggtgttataaccgataaccaggttaagctgatcggtgagacctcaattctaggtagaactgttgttattcacgacggaactgacgatctaggaaagggtggtcacgccgactctttgaagaccggtaacgctggtggaagaccagcttgtggtgtcatcggtttggcagcttaa

SEQ ID NO: 5 - DNA, 465 bp, synthetic construct
  source 1..465: mol_type = other DNA
atggcgacgaaggccgtgtgcgtgctgaagggcgacggcccagtgcagggcatcatcaatttcgagcagaaggaaagtaatggaccagtgaaggtgtggggaagcattaaaggactgactgaaggcctgcatggattccatgttcatgagtttggagataatacagcaggctgtaccagtgcaggtcctcactttaatcctctatccagaaaacacggtgggccaaaggatgaagagaggcatgttggagacttgggcaatgtgactgctgacaaagatggtgtggccgatgtgtctattgaagattctgtgatctcactctcaggagaccattgcatcattggccgcacactggtggtccatgaaaaagcagatgacttgggcaaaggtggaaatgaagaaagtacaaagacaggaaacgctggaagtcgtttggcttgtggtgtaattgggatcgcccaataa

SEQ ID NO: 6 - DNA, 1512 bp, synthetic construct
  source 1..1512: mol_type = other DNA
atgagcgtagaggacagaaaacgtcttgtggacgataatccacctcagccggatcataaaaagcctaagctgccaaaggtactggatcagttgagcgagcctggtgagatgttgacccagaatgacatagtatttttcaagaaggaagcgatatggcgacagatgaatcacttcaaatctaacgtgaatctaatcggttcagagttggaaaagtacaaatctggatatgctaaaagcgtttctcatttgagcacggtcaatgagtggatagaccagcttgttgccgctttcttggagcaaggcttcaaagtatcagatgagataaatgacaaactggtcgtagactttgattgttccccggaccaagaggaaggcgaacatgtaagccaattactggagaagctcagagagaagagaataaccctaatcaagctgtttactcccttgttgaactcgaaactgggtgatacttctgaagacactgcagctttgaaagattctctggctagagcccatagagaaaggagtacgttgattcaggagaataaaatcctgaactcgactcttaaagacattaaacaacaatatcttgatattgtcaaagtaaaggatagactggaatctaaatccttgagtagaataaacgggaacaccgaggaaggtcaaccggcggagaataacatcaaactagagcctagtgatggtaacgactcagaaacaatttccacaacagctgcgaaaacagagacaaatggtactcctgtaaataatgaaacaacagaccatgatgaggatctccagaataatctggaaaaggtaaagctggagaacagcctactattacagcaattgcaagaaacacagcaaaaactatcaataaatgagaagaagctccatgagttgaatcttgtgttgaacaacctatctggggatatgctactaaagaatagtgtggtatatagttctctttattccaattataacgatttggaagcaaaatttaaagagctgcaagatgccgataagcttaacgtggagattgtgtcaaagttacaggccaataatttagattttgagaagaagattgtccaagaattcgaaaaggaaaagaacctgctacagaaacaacttgccaaaaacgaacaagatctggcaagaattagaagtaatagggacgagctgttatctcaggtcagcatgctcaaggctgaaaaggacaaggatctgctgtatcaagagttacaaaagttgattgatattcagaacgctagaatagatcagttatctgcggagaaacaagtgaatgaatttgaggataaaggtgaggacagagatgtattattgaagaaaatccagttactattggcagaattgaaagatattgaagctgttttcaagaagactagagaaatcgaatctgagaaactcaaacaatatgtggactctagttcagtgataacaaagttgaccaccgaaaaaacaaggctgatcagaaatactttgccacaatga

SEQ ID NO: 7 - DNA, 1416 bp, synthetic construct
  source 1..1416: mol_type = other DNA
atgtttgagaagagtaaatttgtggtttcgtttctgcttttactgcagctattttgtgtccttggtgtacatggacaagaaagtggtaacggtaccactagtgacactgcctacgcatgcgacatcggtgcaacaccttttgacggattcaatgctactatttatcagtaccaggcaagtgatgacaattcaatacaggacccggtttttatgagcactgggtacttgcaacgtaaccagttgcatagtacaactggagtgactaatccggggttcaacatcttcactgcaggcgttgccaccacaacactttatgggataccaaacgtcaactaccaaaatatgcttttagaattgaaaggctatttcagagctgacgcctctggaaattatggactatcactaaggaacatcgatgatagtgcgattcttttctttgggagggagactgcgtttgaatgttgcaatgaaaatttgattcccttggacgaagccccaactgattactcactttttaccattaaagaaggggaagcttcaacaaaccccgactcttatacgtacactcaatacttggaggctgggagatactatcccgtaagaactttctttgccaacataagaacgcgtgccgtgttcaactttacgatgacactgccagacgggagtgaactaacagattttcaaaactacatttttcaatttggagctcttaaccaacaacaatgccaagcagaaatagttaccagggaaaattacacaaccaccaccgaaccatggactggtacctttgaagccacgaccacggtgattccaagtggcactgagccaggtaccgtgattgtccagactccttattctactatcgactccacatctacttggaccggtactttcaccactttcaccaccgatgctgatggaagcaccatcgccgttgtgccatcgtcgactattgatgatcactttgcgtcgactgaaactgttttgacagacactgctatttcaactactgttattaccgtgaccagttgtggtaccagtaagtgtaccaagactacagcactaacaggggtgactcagcgaactctcacaatcgatgatagaactactgtcgtgacgacttactgtcctttgccaactgacgttgccactataaaaacagcaagtgttagcggaagtgaggttgtgcaaacaatctacactgcgaaacacagccaggccgtttcttatgttcatccatcaactgttacaatcacaagagaggtatgtgatgcccaaacttgcacgcaggctactattgtgactggagaaattctgcaaactactgttgtggactctggttctacaactgttgttccaaagtatgttccggtggagacgcatgaaccaacatttgaattgagtactctttaa

SEQ ID NO: 8 - DNA, 2421 bp, synthetic construct
  source 1..2421: mol_type = other DNA
atgaacaagccaaacgggtctgaacaacaaccaccgtcacgcggaatgaagcaagagtcaggaggcccagttacttcatctacgacgccgggtaccaatactggcctagaaaactctcattccatgggggcggatatggagcctgatgttggtgctacctctcctcgccatcttcttaatgggtacatttacgattatttagtcaaatctaacatgcaaaatttggctgatcaatttgcccaagagacggagctcttagaaacagacttgacagtaccaatggatacgccttcaggctatcttctagaatggtggatggtattctgggaccttttcaatgcccgcctaaagcaacggggttcacagaaggcccaccagtatattcagttgaacatgctacgacaacagcaacagaggaccatgcgaaatacagcccgtgttcaaaaagtcccgttgaggccacacacccaatcatctccttcaatgtcacagacttttattccacagcagcctcaacagcaagcacagggacaacagcacgcccaggctcaagcccaagtgcaagcacatcagcaagcccaacaccacgcgcaggcacaagtgccagtgcaaccgcaacagcaccagctaggaggccaaactcaacagcagcaatccattaacactgggtctcctgcgggtccaaatgctatcaactcgcgtgttcaacacttagcacaacaacagatgaatcaccttcgccagcaggcgactgccactacgcaacaacctatcccgcaacagaatatcccatcaaaccaacagggtcctacaggcccttatcctacttccccttcaagaagaccgagattactgtctaacgaatcgggtgcaagtgcaccctctgtaatgacaaagtcacagctccaaggagtccctccctcacaacaaccacaccagcagcaaggtcagcaggtaggcccccctaatcaacatcaaggtcaatcttcttccttttattcgggcatgcctcctcaaggggtcgtggttcctcatcagttcaatcctcagcagtatgccaatatgctagcaagacaacagcatgtacaagctcaacaacaggttcagttacaacaggtccaacatgtacaacagagacaacagcaagaccaacaacaacaccgcctgtccgccggttcaccggggcacccttcatttggcgtttttcaacaacctcctccgatgtcaaaccataatcaggtcatgatcaatcagcagggagaaactttttttgatccacattctccatatgctcaacctaacgggtacccccagccacagcaacaacaacaacaacagcaacaacaacaacaacagcagcaaccgcaacagcagcagcagcagcagcagcaacagaagcagcaaccaccaccaccaccacgacagcctcagcgccaacaagcgatggccatggctcctctgcctcactctacttctgccgccggtactcctcactcgtccaccacacctagattctcgcaacctggtcctgtttatcagcagcctttacctgcatctcaaccgcaacattctccgccttcttctattcagcagccggagctagttccaactccagggtcacaacatcagcaaatagcacaaccacaatcacagagccaacaccagcaatcgcaacagtctcaatcaagtgcttctaaaattgtaggtatacaggagtatcagaaagagctaatgatgcttgagaaacagaacaaacagcgtcatgacatggcatgtaagaagggaagcgggcatttttctaactttgatccaattccagagcacacaccgcccgaaccaaaatttaatgtgaatgtaatgctccctccccagaactctgcagtggtcacgaagaatactcccggaacttcacctggtacacaaactcaaaacactgcacatagtactggtaacacttctgcggggtctacaccaaataatgtcgcacctgtacgaaagaaaaaggagccagctaaaaagaaggcaaagaaagctactgagcccccgactcccactactccacagactccaattgcagctaggacacatcaaaactctacaggcggcattcctggtaataatgctgctactaagcgacgaaaacgggagccgctggttgatcaaactgtttcacctaaccttaacgaagcttccaagtcaacaaagaccggaaaaatttcatctcaaactgactttacaggttctgacaatggattcttacaggattttggcgatggaactggtcctcccactggaaccgatgatatggaatttgattttaacagttttcttaataacgaaactggcgaacctaatagttcaaccattcattttgacaatgtattcaattggggagaaggtaccgaagccggagatttatag

SEQ ID NO: 9 - DNA, 2394 bp, synthetic construct
  source 1..2394: mol_type = other DNA
atggtttcactgcgatcgatattcacctcttctatcttagctgcaggtctgacaagagctcatggaagctcaggaaagacttgccctacttctgaggtctctcctgcctgttatgccaatcaatgggaaacaacgtttcctccttccgacataaaaattactggggctacttgggtgcaagacaatatatacgatgtgaccctctcttatgaagcagagtcgttggagttagagaatctgactgagctcaagattattggtcttaacagtcctacaggtggtacaaagctcgtttggtccctaaactcgaaagtatacgacattgacaacccagcaaaatggaccacaactctaagagtttatacaaagagttcagcggatgattgttacgtcgaaatgtacccattccagattcaagttgactggtgtgaagctggtgcttctactgacggatgcagcgcatggaagtggcctaagagttacgactatgatattggatgtgacaacatgcaggacggtgtttcaagaaaacaccaccctaagtgctcctccgactgtggtgttgaaccaactacatctgatgagcctgaagagccaactacatctgaggagcctgtagaaccaacttcctctgatgaagagccaactacctctgaggagccaactacttccgaagagcctgaagagccaaccacttctgatgaacctgaagagccaactacatctgaggagcctgaagagccaaccacttctgaggagcctgaagaaccaaccacttctgaagagccaactacatctgaagagcctgaagagccaacctcctccgatgaggagccaaccacttctgatgaacctgaagagccaactacatctgaggagcctgaagagccaaccacttctgaggagcctgaagaaccaactacttctgaagaacctgaagaaccaactacatctgacgagcctgaagaaccaaccacttctgaggagcctgaagagccaaccacttctgaggagcctgaagaaccaacttcctccgacgaagagccaactacttccgaagagcctgaagagccaaccacttctgaggagcctgaagaaccaactacctctgaggagcctgaagaaccaactacctctgaggagcctgaagaaccaacttcctccgacgaagagccaactacttccgaagagcctgaagagccaaccacttctgatgaacctgaagagccaactacatctgaggagcctgaagagccaaccacttctgaggagcctgaagaaccaacttcctccgacgaagagccaactacttccgaagagcctgaagagccaaccacttctgatgaacctgaagagccaactacatctgaggagcctgaagagccaaccacttctgaggagcctgaagaaccaactacctctgaggagcctgaagaaccaactacctctgaggagcctgaagaaccaacttcctccgacgaagagccaactacttccgaagagcctgaagagccaaccacttctgatgaacctgaagagccaactacatctgaggagcctgaagagccaaccacttctgaggagcctgaagaaccaaccacttctgaggaacctgaagagccaactacctccgatgaggagccaggaactaccgaggagcctttagtgccaactactaagacagaaacggacgtctcaactaccttgttgactgtcactgattgtggaaccaaaacctgcaccaagtctttggtcataactggagttaccaaggagactgtcactactcatggaaaaactactgttataactacttactgtcctttgccaacagaaacagttacgccaaccccagtcaccgttacttctaccatttatgctgacgaaagtgtcactaagaccaccgtctacaccactggtgccgttgagaagacagttaccgttggaggttcttctactgttgtcgtagtccacacaccattgacaactgcagtggtgcaaagccagtccactgatgaaatcaagaccgttgtcactgcccgcccatctaccaccactattgtgagagatgtgtgttacaacagtgtttgctcagttgctacaatagttactggtgtcacagaaaagaccataaccttcagcactggatcaattaccgttgttccaacctatgttccactggtggaatctgaagaacatcaaagaacagcttcaacctctgaaaccagagctaccagtgttgttgtaccaactgttgtaggacaatcatcaagtgcttctgctacttcctccatcttcccatcagtcaccatccatgaaggtgtcgcaaatactgtgaagaattctatgatatccggagcagttgcacttctcttcaatgcattgttcctataa

SEQ ID NO: 10 - DNA, 20 bp, synthetic construct
  source 1..20: mol_type = other DNA
gcacacaagagtgaggttgc

SEQ ID NO: 11 - DNA, 20 bp, synthetic construct
  source 1..20: mol_type = other DNA
caggaccacggatagatagt

SEQ ID NO: 12 - DNA, 20 bp, synthetic construct
  source 1..20: mol_type = other DNA
tggtcaaagcagttgcagtc

SEQ ID NO: 13 - DNA, 20 bp, synthetic construct
  source 1..20: mol_type = other DNA
caaaccgatgacaccacaag

SEQ ID NO: 14 - DNA, 20 bp, synthetic construct
  source 1..20: mol_type = other DNA
ggagataatacagcaggctg

SEQ ID NO: 15 - DNA, 19 bp, synthetic construct
  source 1..19: mol_type = other DNA
cgatcccaattacaccaca

SEQ ID NO: 16 - DNA, 20 bp, synthetic construct
  source 1..20: mol_type = other DNA
ggcgacagatgaatcacttc

SEQ ID NO: 17 - DNA, 20 bp, synthetic construct
  source 1..20: mol_type = other DNA
cacaatctccacgttaagct